European Patent Specification EP 3 950 709 B1, published February 14, 2024. Title: METHODS AND PHARMACEUTICAL COMPOSITIONS FOR PROMOTING T CELLS RESPONSE. Applicant: INSTITUT NATIONAL DE LA SANTE ET DE LA RECHERCHE MEDICALE Université de Nantes OSE Immunotherapeutics. Application EPxxxxxxxx.x. The sequence listing filed with the application follows.

SEQUENCE LISTING (2 sequences)

SEQ ID NO: 1 - protein, 206 aa, Artificial Sequence
  SEQ ID NO:1
YYQLSNTGQDTISQMEERLGNTSQELQSLQVQNIKLAGSLQHVAEKLCRELYNKAGAHRCSPCTEQWKWHGDNCYQFYKDSKSWEDCKYFCLSENSTMLKINKQEDLEFAASQSYSEFFYSYWTGLLRPDSGKAWLWMDGTPFTSELFHIIIDVTSPRSRDCVAILNGMIFSKDCKELKRCVCERRAGMVKPESLHVPPETLGEGD

SEQ ID NO: 2 - protein, 24 aa, Artificial Sequence
  SEQ ID NO:2
CERRAGMVKPESLHVPPETLGEGD